European Patent Specification EP 3 871 696 B1, published March 19, 2025. Title: LIPID FORMULATIONS FOR DELIVERY OF MESSENGER RNA. Applicant: TRANSLATE BIO, INC. MASSACHUSETTS INSTITUTE OF TECHNOLOGY. The sequence listing filed with the application follows.

SEQUENCE LISTING (15 sequences)

SEQ ID NO: 1 - RNA, 1632 nt, Artificial Sequence
  source: /note="Description of Artificial Sequence: Synthetic polynucleotide"
  Variation (1527)..(1527): /replace=" "
  Variation (1627)..(1627): /replace=" "
  misc_feature (1)..(1632): /note="Variant nucleotides given in the sequence have no preference with respect to those in the annotations for variant positions"
ggacagaucgccuggagacgccauccacgcuguuuugaccuccauagaagacaccgggaccgauccagccuccgcggccgggaacggugcauuggaacgcggauuccccgugccaagagugacucaccguccuugacacgaugcagcgcgugaacaugaucauggcagaaucaccaggccucaucaccaucugccuuuuaggauaucuacucagugcugaauguacaguuuuucuugaucaugaaaacgccaacaaaauucugaggcggagaaggagguauaauucagguaaauuggaagaguuuguucaagggaaccuugagagagaauguauggaagaaaaguguaguuuugaagaagcacgagaaguuuuugaaaacacugaaagaacaacugaauuuuggaagcaguauguugauggagaucagugugaguccaauccauguuuaaauggcggcaguugcaaggaugacauuaauuccuaugaauguuggugucccuuuggauuugaaggaaagaacugugaauuagauguaacauguaacauuaagaauggcagaugcgagcaguuuuguaaaaauagugcugauaacaaggugguuugcuccuguacugagggauaucgacuugcagaaaaccagaaguccugugaaccagcagugccauuuccauguggaagaguuucuguuucacaaacuucuaagcucacccgugcugaggcuguuuuuccugauguggacuauguaaauucuacugaagcugaaaccauuuuggauaacaucacucaaagcacccaaucauuuaaugacuucacucggguuguugguggagaagaugccaaaccaggucaauucccuuggcagguuguuuugaaugguaaaguugaugcauucuguggaggcucuaucguuaaugaaaaauggauuguaacugcugcccacuguguugaaacugguguuaaaauuacaguugucgcaggugaacauaauauugaggagacagaacauacagagcaaaagcgaaaugugauucgaauuauuccucaccacaacuacaaugcagcuauuaauaaguacaaccaugacauugcccuucuggaacuggacgaacccuuagugcuaaacagcuacguuacaccuauuugcauugcugacaaggaauacacgaacaucuuccucaaauuuggaucuggcuauguaaguggcuggggaagagucuuccacaaagggagaucagcuuuaguucuucaguaccuuagaguuccacuuguugaccgagccacaugucuucgaucuacaaaguucaccaucuauaacaacauguucugugcuggcuuccaugaaggagguagagauucaugucaaggagauagugggggaccccauguuacugaaguggaagggaccaguuucuuaacuggaauuauuagcuggggugaagagugugcaaugaaaggcaaauauggaauauauaccaagguaucccgguaugucaacuggauuaaggaaaaaacaaagcucacuuaacggguggcaucccugugaccccuccccagugccucuccuggcccuggaaguugccacuccagugcccaccagccuuguccuaauaaaauuaaguugcaucaaagcu

SEQ ID NO: 2 - RNA, 1485 nt, Artificial Sequence
  source: /note="Description of Artificial Sequence: Synthetic polynucleotide"
  Variation (1380)..(1380): /replace=" "
  Variation (1480)..(1480): /replace=" "
  misc_feature (1)..(1485): /note="Variant nucleotides given in the sequence have no preference with respect to those in the annotations for variant positions"
ggacagaucgccuggagacgccauccacgcuguuuugaccuccauagaagacaccgggaccgauccagccuccgcggccgggaacggugcauuggaacgcggauuccccgugccaagagugacucaccguccuugacacgaugagcagcaagggcagcguggugcuggccuacagcggcggccuggacaccagcugcauccugguguggcugaaggagcagggcuacgacgugaucgccuaccuggccaacaucggccagaaggaggacuucgaggaggcccgcaagaaggcccugaagcugggcgccaagaagguguucaucgaggacgugagccgcgaguucguggaggaguucaucuggcccgccauccagagcagcgcccuguacgaggaccgcuaccugcugggcaccagccuggcccgccccugcaucgcccgcaagcagguggagaucgcccagcgcgagggcgccaaguacgugagccacggcgccaccggcaagggcaacgaccaggugcgcuucgagcugagcugcuacagccuggccccccagaucaaggugaucgcccccuggcgcaugcccgaguucuacaaccgcuucaagggccgcaacgaccugauggaguacgccaagcagcacggcauccccauccccgugacccccaagaaccccuggagcauggacgagaaccugaugcacaucagcuacgaggccggcauccuggagaaccccaagaaccaggccccccccggccuguacaccaagacccaggaccccgccaaggcccccaacacccccgacauccuggagaucgaguucaagaagggcgugcccgugaaggugaccaacgugaaggacggcaccacccaccagaccagccuggagcuguucauguaccugaacgagguggccggcaagcacggcgugggccgcaucgacaucguggagaaccgcuucaucggcaugaagagccgcggcaucuacgagacccccgccggcaccauccuguaccacgcccaccuggacaucgaggccuucaccauggaccgcgaggugcgcaagaucaagcagggccugggccugaaguucgccgagcugguguacaccggcuucuggcacagccccgagugcgaguucgugcgccacugcaucgccaagagccaggagcgcguggagggcaaggugcaggugagcgugcugaagggccagguguacauccugggccgcgagagcccccugagccuguacaacgaggagcuggugagcaugaacgugcagggcgacuacgagcccaccgacgccaccggcuucaucaacaucaacagccugcgccugaaggaguaccaccgccugcagagcaaggugaccgccaagugacggguggcaucccugugaccccuccccagugccucuccuggcccuggaaguugccacuccagugcccaccagccuuguccuaauaaaauuaaguugcaucaaagcu

SEQ ID NO: 3 - RNA, 1899 nt, Artificial Sequence
  source: /note="Description of Artificial Sequence: Synthetic polynucleotide"
  Variation (1794)..(1794): /replace=" "
  Variation (1894)..(1894): /replace=" "
  misc_feature (1)..(1899): /note="Variant nucleotides given in the sequence have no preference with respect to those in the annotations for variant positions"
ggacagaucgccuggagacgccauccacgcuguuuugaccuccauagaagacaccgggaccgauccagccuccgcggccgggaacggugcauuggaacgcggauuccccgugccaagagugacucaccguccuugacacgauggaagaugccaaaaacauuaagaagggcccagcgccauucuacccacucgaagacgggaccgccggcgagcagcugcacaaagccaugaagcgcuacgcccuggugcccggcaccaucgccuuuaccgacgcacauaucgagguggacauuaccuacgccgaguacuucgagaugagcguucggcuggcagaagcuaugaagcgcuaugggcugaauacaaaccaucggaucguggugugcagcgagaauagcuugcaguucuucaugcccguguugggugcccuguucaucgguguggcuguggccccagcuaacgacaucuacaacgagcgcgagcugcugaacagcaugggcaucagccagcccaccgucguauucgugagcaagaaagggcugcaaaagauccucaacgugcaaaagaagcuaccgaucauacaaaagaucaucaucauggauagcaagaccgacuaccagggcuuccaaagcauguacaccuucgugacuucccauuugccacccggcuucaacgaguacgacuucgugcccgagagcuucgaccgggacaaaaccaucgcccugaucaugaacaguaguggcaguaccggauugcccaagggcguagcccuaccgcaccgcaccgcuuguguccgauucagucaugcccgcgaccccaucuucggcaaccagaucauccccgacaccgcuauccucagcguggugccauuucaccacggcuucggcauguucaccacgcugggcuacuugaucugcggcuuucgggucgugcucauguaccgcuucgaggaggagcuauucuugcgcagcuugcaagacuauaagauucaaucugcccugcuggugcccacacuauuuagcuucuucgcuaagagcacucucaucgacaaguacgaccuaagcaacuugcacgagaucgccagcggcggggcgccgcucagcaaggagguaggugaggccguggccaaacgcuuccaccuaccaggcauccgccagggcuacggccugacagaaacaaccagcgccauucugaucacccccgaaggggacgacaagccuggcgcaguaggcaagguggugcccuucuucgaggcuaaggugguggacuuggacaccgguaagacacugggugugaaccagcgcggcgagcugugcguccguggccccaugaucaugagcggcuacguuaacaaccccgaggcuacaaacgcucucaucgacaaggacggcuggcugcacagcggcgacaucgccuacugggacgaggacgagcacuucuucaucguggaccggcugaagagccugaucaaauacaagggcuaccagguagccccagccgaacuggagagcauccugcugcaacaccccaacaucuucgacgccggggucgccggccugcccgacgacgaugccggcgagcugcccgccgcagucgucgugcuggaacacgguaaaaccaugaccgagaaggagaucguggacuauguggccagccagguuacaaccgccaagaagcugcgcggugguguuguguucguggacgaggugccuaaaggacugaccggcaaguuggacgcccgcaagauccgcgagauucucauuaaggccaagaagggcggcaagaucgccguguaacggguggcaucccugugaccccuccccagugccucuccuggcccuggaaguugccacuccagugcccaccagccuuguccuaauaaaauuaaguugcaucaaagcu

SEQ ID NO: 4 - RNA, 1131 nt, Artificial Sequence
  source: /note="Description of Artificial Sequence: Synthetic polynucleotide"
  Variation (1026)..(1026): /replace=" "
  Variation (1126)..(1126): /replace=" "
  misc_feature (1)..(1131): /note="Variant nucleotides given in the sequence have no preference with respect to those in the annotations for variant positions"
ggacagaucgccuggagacgccauccacgcuguuuugaccuccauagaagacaccgggaccgauccagccuccgcggccgggaacggugcauuggaacgcggauuccccgugccaagagugacucaccguccuugacacgauggccaugagcagcggaggcagcggcggaggagugcccgagcaggaggacagcgugcuguucaggagaggcaccggccagagcgaugacagcgauaucugggacgauaccgcucugaucaaggccuacgacaaggccguggccagcuucaagcacgcccugaaaaacggcgacaucugcgagaccagcggcaagcccaagacaacccccaagagaaagcccgccaagaagaauaagagccagaaaaagaacaccgccgccagccugcagcaguggaaggugggcgacaagugcagcgccaucuggagcgaggacggcugcaucuaccccgccaccaucgccagcaucgacuucaagagagagaccugcguggucguguacaccggcuacggcaacagagaggagcagaaccugagcgaccugcugagccccauuugugagguggccaauaacaucgaacagaacgcccaggagaacgagaaugaaagccaggugagcaccgacgagagcgagaacagcagaucuccuggcaacaagagcgacaacaucaagccuaagucugccccuuggaacagcuuccugcccccuccuccacccaugcccggacccagacugggacccggaaaaccuggccugaaguucaacggaccaccucccccuccaccuccucccccaccucaucuccugagcugcuggcugccacccuuccccagcggacccccuaucaucccaccacccccucccaucugccccgacagccuggacgacgccgaugcccugggcagcaugcugaucagcugguacaugagcggcuaccacacaggauacuacaugggcuucagacagaaccagaaggagggcagaugcucccacucccugaacugacggguggcaucccugugaccccuccccagugccucuccuggcccuggaaguugccacuccagugcccaccagccuuguccuaauaaaauuaaguugcaucaaagcu

SEQ ID NO: 5 - RNA, 140 nt, Artificial Sequence
  source: /note="Description of Artificial Sequence: Synthetic polynucleotide"
ggacagaucgccuggagacgccauccacgcuguuuugaccuccauagaagacaccgggaccgauccagccuccgcggccgggaacggugcauuggaacgcggauuccccgugccaagagugacucaccguccuugacacg

SEQ ID NO: 6 - RNA, 105 nt, Artificial Sequence
  source: /note="Description of Artificial Sequence: Synthetic polynucleotide"
cggguggcaucccugugaccccuccccagugccucuccuggcccuggaaguugccacuccagugcccaccagccuuguccuaauaaaauuaaguugcaucaagcu

SEQ ID NO: 7 - RNA, 105 nt, Artificial Sequence
  source: /note="Description of Artificial Sequence: Synthetic polynucleotide"
ggguggcaucccugugaccccuccccagugccucuccuggcccuggaaguugccacuccagugcccaccagccuuguccuaauaaaauuaaguugcaucaaagcu

SEQ ID NO: 8 - RNA, 4719 nt, Artificial Sequence
  source: /note="Description of Artificial Sequence: Synthetic polynucleotide"
  Variation (4614)..(4614): /replace=" "
  Variation (4714)..(4714): /replace=" "
  misc_feature (1)..(4719): /note="Variant nucleotides given in the sequence have no preference with respect to those in the annotations for variant positions"
ggacagaucgccuggagacgccauccacgcuguuuugaccuccauagaagacaccgggaccgauccagccuccgcggccgggaacggugcauuggaacgcggauuccccgugccaagagugacucaccguccuugacacgaugcagcgguccccgcucgaaaaggccagugucguguccaaacucuucuucucauggacucggccuauccuuagaaagggguaucggcagaggcuugaguugucugacaucuaccagauccccucgguagauucggcggauaaccucucggagaagcucgaacgggaaugggaccgcgaacucgcgucuaagaaaaacccgaagcucaucaacgcacugagaaggugcuucuucuggcgguucauguucuacgguaucuucuuguaucucggggaggucacaaaagcaguccaaccccuguuguugggucgcauuaucgccucguacgaccccgauaacaaagaagaacggagcaucgcgaucuaccucgggaucggacuguguuugcuuuucaucgucagaacacuuuuguugcauccagcaaucuucggccuccaucacaucgguaugcagaugcgaaucgcuauguuuagcuugaucuacaaaaagacacugaaacucucgucgcggguguuggauaagauuuccaucggucaguuggugucccugcuuaguaauaaccucaacaaauucgaugagggacuggcgcuggcacauuucguguggauugccccguugcaagucgcccuuuugaugggccuuauuugggagcuguugcaggcaucugccuuuuguggccugggauuucugauuguguuggcauuguuucaggcugggcuugggcggaugaugaugaaguaucgcgaccagagagcggguaaaaucucggaaagacucgucaucacuucggaaaugaucgaaaacauccagucggucaaagccuauugcugggaagaagcuauggagaagaugauugaaaaccuccgccaaacugagcugaaacugacccgcaaggcggcguauguccgguauuucaauucgucagcguucuucuuuuccggguucuucguugucuuucucucgguuuugccuuaugccuugauuaaggggauuauccuccgcaagauuuucaccacgauuucguucugcauuguauugcgcauggcagugacacggcaauuuccgugggccgugcagacaugguaugacucgcuuggagcgaucaacaaaauccaagacuucuugcaaaagcaagaguacaagacccuggaguacaaucuuacuacuacggagguaguaauggagaaugugacggcuuuuugggaagaggguuuuggagaacuguuugagaaagcaaagcagaauaacaacaaccgcaagaccucaaauggggacgauucccuguuuuucucgaacuucucccugcucggaacacccguguugaaggacaucaauuucaagauugagaggggacagcuucucgcgguagcgggaagcacuggugcgggaaaaacuagccucuugauggugauuaugggggagcuugagcccagcgaggggaagauuaaacacuccgggcguaucucauucuguagccaguuuucauggaucaugcccggaaccauuaaagagaacaucauuuucggaguauccuaugaugaguaccgauacagaucggucauuaaggcgugccaguuggaagaggacauuucuaaguucgccgagaaggauaacaucgucuugggagaaggggguauuacauugucgggagggcagcgagcgcggaucagccucgcgagagcgguauacaaagaugcagauuuguaucugcuugauucaccguuuggauaccucgacguauugacagaaaaagaaaucuucgagucgugcguguguaaacuuauggcuaauaagacgagaauccuggugacaucaaaaauggaacaccuuaagaaggcggacaagauccugauccuccacgaaggaucguccuacuuuuacggcacuuucucagaguugcaaaacuugcagccggacuucucaagcaaacucauggggugugacucauucgaccaguucagcgcggaacggcggaacucgaucuugacggaaacgcugcaccgauucucgcuugagggugaugccccgguaucguggaccgagacaaagaagcagucguuuaagcagacaggagaauuuggugagaaaagaaagaacaguaucuugaauccuauuaacucaauucgcaaguucucaaucguccagaaaacuccacugcagaugaauggaauugaagaggauucggacgaaccccuggagcgcaggcuuagccucgugccggauucagagcaaggggaggccauucuuccccggauuucggugauuucaaccggaccuacacuucaggcgaggcgaaggcaauccgugcucaaccucaugacgcauucgguaaaccaggggcaaaacauucaccgcaaaacgacggccucaacgagaaaagugucacuugcaccccaggcgaauuugacugaacucgacaucuacagccguaggcuuucgcaagaaaccggacuugagaucagcgaagaaaucaaugaagaagauuugaaagaguguuucuuugaugacauggaaucaaucccagcggugacaacguggaacacauacuugcguuacaucacggugcacaaguccuugauuuucguccucaucuggugucucgugaucuuucucgcugaggucgcagcgucacuugugguccucuggcugcuugguaauacgcccuugcaagacaaaggcaauucuacacacucaagaaacaauuccuaugccgugauuaucacuucuacaagcucguauuacguguuuuacaucuacguaggaguggccgacacucugcucgcgauggguuucuuccgaggacucccacucguucacacgcuuaucacugucuccaagauucuccaccauaagaugcuucauagcguacugcaggcucccauguccaccuugaauacgcucaaggcgggagguauuuugaaucgcuucucaaaagauauugcaauuuuggaugaccuucugccccugacgaucuucgacuucauccaguuguugcugaucgugauuggggcuauugcaguagucgcuguccuccagccuuacauuuuugucgcgaccguuccggugaucguggcguuuaucaugcugcgggccuauuucuugcagacgucacagcagcuuaagcaacuggagucugaagggaggucgccuaucuuuacgcaucuugugaccaguuugaagggauuguggacguugcgcgccuuuggcaggcagcccuacuuugaaacacuguuccacaaagcgcugaaucuccauacggcaaauugguuuuuguauuugaguacccuccgaugguuucagaugcgcauugagaugauuuuugugaucuucuuuaucgcggugacuuuuaucuccaucuugaccacgggagagggcgagggacgggucgguauuauccugacacucgccaugaacauuaugagcacuuugcagugggcagugaacagcucgauugauguggauagccugaugagguccguuucgagggucuuuaaguucaucgacaugccgacggagggaaagcccacaaaaaguacgaaacccuauaagaaugggcaauugaguaagguaaugaucaucgagaacagucacgugaagaaggaugacaucuggccuagcgggggucagaugaccgugaaggaccugacggcaaaauacaccgagggagggaacgcaauccuugaaaacaucucguucagcauuagccccggucagcgugugggguugcucgggaggaccgggucaggaaaaucgacguugcugucggccuucuugagacuucugaauacagagggugagauccagaucgacggcguuucgugggauagcaucaccuugcagcaguggcggaaagcguuuggaguaaucccccaaaaggucuuuaucuuuagcggaaccuuccgaaagaaucucgauccuuaugaacaguggucagaucaagagauuuggaaagucgcggacgagguuggccuucggaguguaaucgagcaguuuccgggaaaacucgacuuuguccuuguagaugggggaugcguccugucgcaugggcacaagcagcucaugugccuggcgcgauccguccucucuaaagcgaaaauucuucucuuggaugaaccuucggcccaucuggacccgguaacguaucagaucaucagaaggacacuuaagcaggcguuugccgacugcacggugauucucugugagcaucguaucgaggccaugcucgaaugccagcaauuucuugucaucgaagagaauaagguccgccaguacgacuccauccagaagcugcuuaaugagagaucauuguuccggcaggcgauuucaccauccgauagggugaaacuuuuuccacacagaaauucgucgaagugcaaguccaaaccgcagaucgcggccuugaaagaagagacugaagaagaaguucaagacacgcgucuucaccaucaccaucaccaucaccaucaccauuaacggguggcaucccugugaccccuccccagugccucuccuggcccuggaaguugccacuccagugcccaccagccuuguccuaauaaaauuaaguugcaucaaagcu

SEQ ID NO: 9 - RNA, 4689 nt, Artificial Sequence
  source: /note="Description of Artificial Sequence: Synthetic polynucleotide"
  Variation (4584)..(4584): /replace=" "
  Variation (4684)..(4684): /replace=" "
  misc_feature (1)..(4689): /note="Variant nucleotides given in the sequence have no preference with respect to those in the annotations for variant positions"
ggacagaucgccuggagacgccauccacgcuguuuugaccuccauagaagacaccgggaccgauccagccuccgcggccgggaacggugcauuggaacgcggauuccccgugccaagagugacucaccguccuugacacgaugcagcgguccccgcucgaaaaggccagugucguguccaaacucuucuucucauggacucggccuauccuuagaaagggguaucggcagaggcuugaguugucugacaucuaccagauccccucgguagauucggcggauaaccucucggagaagcucgaacgggaaugggaccgcgaacucgcgucuaagaaaaacccgaagcucaucaacgcacugagaaggugcuucuucuggcgguucauguucuacgguaucuucuuguaucucggggaggucacaaaagcaguccaaccccuguuguugggucgcauuaucgccucguacgaccccgauaacaaagaagaacggagcaucgcgaucuaccucgggaucggacuguguuugcuuuucaucgucagaacacuuuuguugcauccagcaaucuucggccuccaucacaucgguaugcagaugcgaaucgcuauguuuagcuugaucuacaaaaagacacugaaacucucgucgcggguguuggauaagauuuccaucggucaguuggugucccugcuuaguaauaaccucaacaaauucgaugagggacuggcgcuggcacauuucguguggauugccccguugcaagucgcccuuuugaugggccuuauuugggagcuguugcaggcaucugccuuuuguggccugggauuucugauuguguuggcauuguuucaggcugggcuugggcggaugaugaugaaguaucgcgaccagagagcggguaaaaucucggaaagacucgucaucacuucggaaaugaucgaaaacauccagucggucaaagccuauugcugggaagaagcuauggagaagaugauugaaaaccuccgccaaacugagcugaaacugacccgcaaggcggcguauguccgguauuucaauucgucagcguucuucuuuuccggguucuucguugucuuucucucgguuuugccuuaugccuugauuaaggggauuauccuccgcaagauuuucaccacgauuucguucugcauuguauugcgcauggcagugacacggcaauuuccgugggccgugcagacaugguaugacucgcuuggagcgaucaacaaaauccaagacuucuugcaaaagcaagaguacaagacccuggaguacaaucuuacuacuacggagguaguaauggagaaugugacggcuuuuugggaagaggguuuuggagaacuguuugagaaagcaaagcagaauaacaacaaccgcaagaccucaaauggggacgauucccuguuuuucucgaacuucucccugcucggaacacccguguugaaggacaucaauuucaagauugagaggggacagcuucucgcgguagcgggaagcacuggugcgggaaaaacuagccucuugauggugauuaugggggagcuugagcccagcgaggggaagauuaaacacuccgggcguaucucauucuguagccaguuuucauggaucaugcccggaaccauuaaagagaacaucauuuucggaguauccuaugaugaguaccgauacagaucggucauuaaggcgugccaguuggaagaggacauuucuaaguucgccgagaaggauaacaucgucuugggagaaggggguauuacauugucgggagggcagcgagcgcggaucagccucgcgagagcgguauacaaagaugcagauuuguaucugcuugauucaccguuuggauaccucgacguauugacagaaaaagaaaucuucgagucgugcguguguaaacuuauggcuaauaagacgagaauccuggugacaucaaaaauggaacaccuuaagaaggcggacaagauccugauccuccacgaaggaucguccuacuuuuacggcacuuucucagaguugcaaaacuugcagccggacuucucaagcaaacucauggggugugacucauucgaccaguucagcgcggaacggcggaacucgaucuugacggaaacgcugcaccgauucucgcuugagggugaugccccgguaucguggaccgagacaaagaagcagucguuuaagcagacaggagaauuuggugagaaaagaaagaacaguaucuugaauccuauuaacucaauucgcaaguucucaaucguccagaaaacuccacugcagaugaauggaauugaagaggauucggacgaaccccuggagcgcaggcuuagccucgugccggauucagagcaaggggaggccauucuuccccggauuucggugauuucaaccggaccuacacuucaggcgaggcgaaggcaauccgugcucaaccucaugacgcauucgguaaaccaggggcaaaacauucaccgcaaaacgacggccucaacgagaaaagugucacuugcaccccaggcgaauuugacugaacucgacaucuacagccguaggcuuucgcaagaaaccggacuugagaucagcgaagaaaucaaugaagaagauuugaaagaguguuucuuugaugacauggaaucaaucccagcggugacaacguggaacacauacuugcguuacaucacggugcacaaguccuugauuuucguccucaucuggugucucgugaucuuucucgcugaggucgcagcgucacuugugguccucuggcugcuugguaauacgcccuugcaagacaaaggcaauucuacacacucaagaaacaauuccuaugccgugauuaucacuucuacaagcucguauuacguguuuuacaucuacguaggaguggccgacacucugcucgcgauggguuucuuccgaggacucccacucguucacacgcuuaucacugucuccaagauucuccaccauaagaugcuucauagcguacugcaggcucccauguccaccuugaauacgcucaaggcgggagguauuuugaaucgcuucucaaaagauauugcaauuuuggaugaccuucugccccugacgaucuucgacuucauccaguuguugcugaucgugauuggggcuauugcaguagucgcuguccuccagccuuacauuuuugucgcgaccguuccggugaucguggcguuuaucaugcugcgggccuauuucuugcagacgucacagcagcuuaagcaacuggagucugaagggaggucgccuaucuuuacgcaucuugugaccaguuugaagggauuguggacguugcgcgccuuuggcaggcagcccuacuuugaaacacuguuccacaaagcgcugaaucuccauacggcaaauugguuuuuguauuugaguacccuccgaugguuucagaugcgcauugagaugauuuuugugaucuucuuuaucgcggugacuuuuaucuccaucuugaccacgggagagggcgagggacgggucgguauuauccugacacucgccaugaacauuaugagcacuuugcagugggcagugaacagcucgauugauguggauagccugaugagguccguuucgagggucuuuaaguucaucgacaugccgacggagggaaagcccacaaaaaguacgaaacccuauaagaaugggcaauugaguaagguaaugaucaucgagaacagucacgugaagaaggaugacaucuggccuagcgggggucagaugaccgugaaggaccugacggcaaaauacaccgagggagggaacgcaauccuugaaaacaucucguucagcauuagccccggucagcgugugggguugcucgggaggaccgggucaggaaaaucgacguugcugucggccuucuugagacuucugaauacagagggugagauccagaucgacggcguuucgugggauagcaucaccuugcagcaguggcggaaagcguuuggaguaaucccccaaaaggucuuuaucuuuagcggaaccuuccgaaagaaucucgauccuuaugaacaguggucagaucaagagauuuggaaagucgcggacgagguuggccuucggaguguaaucgagcaguuuccgggaaaacucgacuuuguccuuguagaugggggaugcguccugucgcaugggcacaagcagcucaugugccuggcgcgauccguccucucuaaagcgaaaauucuucucuuggaugaaccuucggcccaucuggacccgguaacguaucagaucaucagaaggacacuuaagcaggcguuugccgacugcacggugauucucugugagcaucguaucgaggccaugcucgaaugccagcaauuucuugucaucgaagagaauaagguccgccaguacgacuccauccagaagcugcuuaaugagagaucauuguuccggcaggcgauuucaccauccgauagggugaaacuuuuuccacacagaaauucgucgaagugcaaguccaaaccgcagaucgcggccuugaaagaagagacugaagaagaaguucaagacacgcgucuuuaacggguggcaucccugugaccccuccccagugccucuccuggcccuggaaguugccacuccagugcccaccagccuuguccuaauaaaauuaaguugcaucaaagcu

SEQ ID NO: 10 - RNA, 4542 nt, Artificial Sequence
  source: /note="Description of Artificial Sequence: Synthetic polynucleotide"
auggccacuggaucaagaaccucacugcugcucgcuuuuggacugcuuugccugcccugguugcaagaaggaucggcuuucccgaccaucccacucuccaugcagcgguccccgcucgaaaaggccagugucguguccaaacucuucuucucauggacucggccuauccuuagaaagggguaucggcagaggcuugaguugucugacaucuaccagauccccucgguagauucggcggauaaccucucggagaagcucgaacgggaaugggaccgcgaacucgcgucuaagaaaaacccgaagcucaucaacgcacugagaaggugcuucuucuggcgguucauguucuacgguaucuucuuguaucucggggaggucacaaaagcaguccaaccccuguuguugggucgcauuaucgccucguacgaccccgauaacaaagaagaacggagcaucgcgaucuaccucgggaucggacuguguuugcuuuucaucgucagaacacuuuuguugcauccagcaaucuucggccuccaucacaucgguaugcagaugcgaaucgcuauguuuagcuugaucuacaaaaagacacugaaacucucgucgcggguguuggauaagauuuccaucggucaguuggugucccugcuuaguaauaaccucaacaaauucgaugagggacuggcgcuggcacauuucguguggauugccccguugcaagucgcccuuuugaugggccuuauuugggagcuguugcaggcaucugccuuuuguggccugggauuucugauuguguuggcauuguuucaggcugggcuugggcggaugaugaugaaguaucgcgaccagagagcggguaaaaucucggaaagacucgucaucacuucggaaaugaucgaaaacauccagucggucaaagccuauugcugggaagaagcuauggagaagaugauugaaaaccuccgccaaacugagcugaaacugacccgcaaggcggcguauguccgguauuucaauucgucagcguucuucuuuuccggguucuucguugucuuucucucgguuuugccuuaugccuugauuaaggggauuauccuccgcaagauuuucaccacgauuucguucugcauuguauugcgcauggcagugacacggcaauuuccgugggccgugcagacaugguaugacucgcuuggagcgaucaacaaaauccaagacuucuugcaaaagcaagaguacaagacccuggaguacaaucuuacuacuacggagguaguaauggagaaugugacggcuuuuugggaagaggguuuuggagaacuguuugagaaagcaaagcagaauaacaacaaccgcaagaccucaaauggggacgauucccuguuuuucucgaacuucucccugcucggaacacccguguugaaggacaucaauuucaagauugagaggggacagcuucucgcgguagcgggaagcacuggugcgggaaaaacuagccucuugauggugauuaugggggagcuugagcccagcgaggggaagauuaaacacuccgggcguaucucauucuguagccaguuuucauggaucaugcccggaaccauuaaagagaacaucauuuucggaguauccuaugaugaguaccgauacagaucggucauuaaggcgugccaguuggaagaggacauuucuaaguucgccgagaaggauaacaucgucuugggagaaggggguauuacauugucgggagggcagcgagcgcggaucagccucgcgagagcgguauacaaagaugcagauuuguaucugcuugauucaccguuuggauaccucgacguauugacagaaaaagaaaucuucgagucgugcguguguaaacuuauggcuaauaagacgagaauccuggugacaucaaaaauggaacaccuuaagaaggcggacaagauccugauccuccacgaaggaucguccuacuuuuacggcacuuucucagaguugcaaaacuugcagccggacuucucaagcaaacucauggggugugacucauucgaccaguucagcgcggaacggcggaacucgaucuugacggaaacgcugcaccgauucucgcuugagggugaugccccgguaucguggaccgagacaaagaagcagucguuuaagcagacaggagaauuuggugagaaaagaaagaacaguaucuugaauccuauuaacucaauucgcaaguucucaaucguccagaaaacuccacugcagaugaauggaauugaagaggauucggacgaaccccuggagcgcaggcuuagccucgugccggauucagagcaaggggaggccauucuuccccggauuucggugauuucaaccggaccuacacuucaggcgaggcgaaggcaauccgugcucaaccucaugacgcauucgguaaaccaggggcaaaacauucaccgcaaaacgacggccucaacgagaaaagugucacuugcaccccaggcgaauuugacugaacucgacaucuacagccguaggcuuucgcaagaaaccggacuugagaucagcgaagaaaucaaugaagaagauuugaaagaguguuucuuugaugacauggaaucaaucccagcggugacaacguggaacacauacuugcguuacaucacggugcacaaguccuugauuuucguccucaucuggugucucgugaucuuucucgcugaggucgcagcgucacuugugguccucuggcugcuugguaauacgcccuugcaagacaaaggcaauucuacacacucaagaaacaauuccuaugccgugauuaucacuucuacaagcucguauuacguguuuuacaucuacguaggaguggccgacacucugcucgcgauggguuucuuccgaggacucccacucguucacacgcuuaucacugucuccaagauucuccaccauaagaugcuucauagcguacugcaggcucccauguccaccuugaauacgcucaaggcgggagguauuuugaaucgcuucucaaaagauauugcaauuuuggaugaccuucugccccugacgaucuucgacuucauccaguuguugcugaucgugauuggggcuauugcaguagucgcuguccuccagccuuacauuuuugucgcgaccguuccggugaucguggcguuuaucaugcugcgggccuauuucuugcagacgucacagcagcuuaagcaacuggagucugaagggaggucgccuaucuuuacgcaucuugugaccaguuugaagggauuguggacguugcgcgccuuuggcaggcagcccuacuuugaaacacuguuccacaaagcgcugaaucuccauacggcaaauugguuuuuguauuugaguacccuccgaugguuucagaugcgcauugagaugauuuuugugaucuucuuuaucgcggugacuuuuaucuccaucuugaccacgggagagggcgagggacgggucgguauuauccugacacucgccaugaacauuaugagcacuuugcagugggcagugaacagcucgauugauguggauagccugaugagguccguuucgagggucuuuaaguucaucgacaugccgacggagggaaagcccacaaaaaguacgaaacccuauaagaaugggcaauugaguaagguaaugaucaucgagaacagucacgugaagaaggaugacaucuggccuagcgggggucagaugaccgugaaggaccugacggcaaaauacaccgagggagggaacgcaauccuugaaaacaucucguucagcauuagccccggucagcgugugggguugcucgggaggaccgggucaggaaaaucgacguugcugucggccuucuugagacuucugaauacagagggugagauccagaucgacggcguuucgugggauagcaucaccuugcagcaguggcggaaagcguuuggaguaaucccccaaaaggucuuuaucuuuagcggaaccuuccgaaagaaucucgauccuuaugaacaguggucagaucaagagauuuggaaagucgcggacgagguuggccuucggaguguaaucgagcaguuuccgggaaaacucgacuuuguccuuguagaugggggaugcguccugucgcaugggcacaagcagcucaugugccuggcgcgauccguccucucuaaagcgaaaauucuucucuuggaugaaccuucggcccaucuggacccgguaacguaucagaucaucagaaggacacuuaagcaggcguuugccgacugcacggugauucucugugagcaucguaucgaggccaugcucgaaugccagcaauuucuugucaucgaagagaauaagguccgccaguacgacuccauccagaagcugcuuaaugagagaucauuguuccggcaggcgauuucaccauccgauagggugaaacuuuuuccacacagaaauucgucgaagugcaaguccaaaccgcagaucgcggccuugaaagaagagacugaagaagaaguucaagacacgcgucuuuaa

SEQ ID NO: 11 - protein, 10 aa, Artificial Sequence
  source: /note="Description of Artificial Sequence: Synthetic 10xHis tag"
HHHHHHHHHH

SEQ ID NO: 12 - DNA, 500 bp, Artificial Sequence
  source: /note="Description of Artificial Sequence: Synthetic polynucleotide"
  misc_feature (1)..(500): /note="This sequence may encompass 10-500 nucleotides"
  Variation (11)..(500): /replace=" "
  misc_feature (1)..(500): /note="Variant nucleotides given in the sequence have no preference with respect to those in the annotations for variant positions"
  source: /note="See specification as filed for detailed description of substitutions and preferred embodiments"
aaaaaaaaaaaaaaaaaaaaaaaaaaaaaaaaaaaaaaaaaaaaaaaaaaaaaaaaaaaaaaaaaaaaaaaaaaaaaaaaaaaaaaaaaaaaaaaaaaaaaaaaaaaaaaaaaaaaaaaaaaaaaaaaaaaaaaaaaaaaaaaaaaaaaaaaaaaaaaaaaaaaaaaaaaaaaaaaaaaaaaaaaaaaaaaaaaaaaaaaaaaaaaaaaaaaaaaaaaaaaaaaaaaaaaaaaaaaaaaaaaaaaaaaaaaaaaaaaaaaaaaaaaaaaaaaaaaaaaaaaaaaaaaaaaaaaaaaaaaaaaaaaaaaaaaaaaaaaaaaaaaaaaaaaaaaaaaaaaaaaaaaaaaaaaaaaaaaaaaaaaaaaaaaaaaaaaaaaaaaaaaaaaaaaaaaaaaaaaaaaaaaaaaaaaaaaaaaaaaaaaaaaaaaaaaaaaaaaaaaaaaaaaaaaaaaaaaaaaaaaaaaaaaaaaaaaaaaaaaaaaaaaaaaaaaaaaaaaaaa

SEQ ID NO: 13 - DNA, 300 bp, Artificial Sequence
  source: /note="Description of Artificial Sequence: Synthetic polynucleotide"
  misc_feature (1)..(300): /note="This sequence may encompass 10-300 nucleotides"
  Variation (11)..(300): /replace=" "
  misc_feature (1)..(300): /note="Variant nucleotides given in the sequence have no preference with respect to those in the annotations for variant positions"
  source: /note="See specification as filed for detailed description of substitutions and preferred embodiments"
aaaaaaaaaaaaaaaaaaaaaaaaaaaaaaaaaaaaaaaaaaaaaaaaaaaaaaaaaaaaaaaaaaaaaaaaaaaaaaaaaaaaaaaaaaaaaaaaaaaaaaaaaaaaaaaaaaaaaaaaaaaaaaaaaaaaaaaaaaaaaaaaaaaaaaaaaaaaaaaaaaaaaaaaaaaaaaaaaaaaaaaaaaaaaaaaaaaaaaaaaaaaaaaaaaaaaaaaaaaaaaaaaaaaaaaaaaaaaaaaaaaaaaaaaaaaaaaaaaaaaaaaaaaaaaaaaaaaaaaaaaaaaaaaaaaaaaaaaaaa

SEQ ID NO: 14 - DNA, 200 bp, Artificial Sequence
  source: /note="Description of Artificial Sequence: Synthetic polynucleotide"
  misc_feature (1)..(200): /note="This sequence may encompass 10-200 nucleotides"
  Variation (11)..(200): /replace=" "
  misc_feature (1)..(200): /note="Variant nucleotides given in the sequence have no preference with respect to those in the annotations for variant positions"
  source: /note="See specification as filed for detailed description of substitutions and preferred embodiments"
cccccccccccccccccccccccccccccccccccccccccccccccccccccccccccccccccccccccccccccccccccccccccccccccccccccccccccccccccccccccccccccccccccccccccccccccccccccccccccccccccccccccccccccccccccccccccccccccccccccccc

SEQ ID NO: 15 - DNA, 250 bp, Artificial Sequence
  source: /note="Description of Artificial Sequence: Synthetic polynucleotide"
  source: /note="See specification as filed for detailed description of substitutions and preferred embodiments"
aaaaaaaaaaaaaaaaaaaaaaaaaaaaaaaaaaaaaaaaaaaaaaaaaaaaaaaaaaaaaaaaaaaaaaaaaaaaaaaaaaaaaaaaaaaaaaaaaaaaaaaaaaaaaaaaaaaaaaaaaaaaaaaaaaaaaaaaaaaaaaaaaaaaaaaaaaaaaaaaaaaaaaaaaaaaaaaaaaaaaaaaaaaaaaaaaaaaaaaaaaaaaaaaaaaaaaaaaaaaaaaaaaaaaaaaaaaaaaaaaaaaaaaaaa